European Patent Specification EP 3 429 618 B1, published February 21, 2024. Title: COMBINATION OF AN IMMUNE CHECKPOINT MODULATOR AND A COMPLEX COMPRISING A CELL PENETRATING PEPTIDE, A CARGO AND A TLR PEPTIDE AGONIST FOR USE IN MEDICINE. Applicant: Amal Therapeutics SA, Geneva, Switzerland. The sequence listing filed with the application follows.

SEQUENCE LISTING (47 sequences)

SEQ ID NO: 1 - protein, 16 aa, Artificial Sequence
  CPP: Penetratin
RQIKIYFQNRRMKWKK

SEQ ID NO: 2 - protein, 11 aa, Artificial Sequence
  CPP: TAT minimal domain
YGRKKRRQRRR

SEQ ID NO: 3 - protein, 245 aa, Artificial Sequence
  ZEBRA amino acid sequence (natural sequence from Epstein - Barr virus (EBV)) (YP_401673)
MMDPNSTSEDVKFTPDPYQVPFVQAFDQATRVYQDLGGPSQAPLPCVLWPVLPEPLPQGQLTAYHVSTAPTGSWFSAPQPAPENAYQAYAAPQLFPVSDITQNQQTNQAGGEAPQPGDNSTVQTAAAVVFACPGANQGQQLADIGVPQPAPVAAPARRTRKPQQPESLEECDSELEIKRYKNRVASRKCRAKFKQLLQHYREVAAAKSSENDRLRLLLKQMCPSLDVDSIIPRTPDVLHEDLLNF

SEQ ID NO: 4 - protein, 45 aa, Artificial Sequence
  CPP1 (Z11)
KRYKNRVASRKCRAKFKQLLQHYREVAAAKSSENDRLRLLLKQMC

SEQ ID NO: 5 - protein, 42 aa, Artificial Sequence
  CPP2 (Z12)
KRYKNRVASRKCRAKFKQLLQHYREVAAAKSSENDRLRLLLK

SEQ ID NO: 6 - protein, 42 aa, Artificial Sequence
  CPP3 (Z13)
KRYKNRVASRKSRAKFKQLLQHYREVAAAKSSENDRLRLLLK

SEQ ID NO: 7 - protein, 30 aa, Artificial Sequence
  CPP4 (Z14)
KRYKNRVASRKSRAKFKQLLQHYREVAAAK

SEQ ID NO: 8 - protein, 17 aa, Artificial Sequence
  CPP5 (Z15)
KRYKNRVASRKSRAKFK

SEQ ID NO: 9 - protein, 15 aa, Artificial Sequence
  CPP6 (Z16)
QHYREVAAAKSSEND

SEQ ID NO: 10 - protein, 13 aa, Artificial Sequence
  CPP7 (Z17)
QLLQHYREVAAAK

SEQ ID NO: 11 - protein, 19 aa, Artificial Sequence
  CPP8 (Z18)
REVAAAKSSENDRLRLLLK

SEQ ID NO: 12 - protein, 8 aa, Artificial Sequence
  CPP9 (Z19)
KRYKNRVA

SEQ ID NO: 13 - protein, 11 aa, Artificial Sequence
  CPP10 (Z20)
VASRKSRAKFK

SEQ ID NO: 14 - protein, 85 aa, Artificial Sequence
  MAD5 cargo
ESLKISQAVHAAHAEINEAGREVVGVGALKVPRNQDWLGVPRFAKFASFEAQGALANIAVDKANLDVEQLESIINFEKLTEWTGS

SEQ ID NO: 15 - protein, 35 aa, Artificial Sequence
  TLR2 peptide agonist Anaxa
STVHEILCKLSLEGDHSTPPSAYGSVKPYTNFDAE

SEQ ID NO: 16 - protein, 4 aa, Artificial Sequence
  enterokinase target site
DDDK

SEQ ID NO: 17 - protein, 5 aa, Artificial Sequence
  factor Xa target site
IEDGR

SEQ ID NO: 18 - protein, 6 aa, Artificial Sequence
  thrombin target site
LVPRGS

SEQ ID NO: 19 - protein, 7 aa, Artificial Sequence
  protease TEV target site
ENLYFQG

SEQ ID NO: 20 - protein, 8 aa, Artificial Sequence
  PreScission protease target site
LEVLFQGP

SEQ ID NO: 21 - protein, 4 aa, Artificial Sequence
  furin target site
  MISC_FEATURE (2)..(2): X may be any amino acid
  MISC_FEATURE (3)..(3): X is R or K
RXXR

SEQ ID NO: 22 - protein, 5 aa, Artificial Sequence
  peptidic linker
GGGGG

SEQ ID NO: 23 - protein, 4 aa, Artificial Sequence
  peptidic linker
GGGG

SEQ ID NO: 24 - protein, 4 aa, Artificial Sequence
  peptidic linker
EQLE

SEQ ID NO: 25 - protein, 4 aa, Artificial Sequence
  peptidic linker
TEWT

SEQ ID NO: 26 - protein, 224 aa, Artificial Sequence
  EDAZ13Mad5
MHHHHHHNIDRPKGLAFTDVDVDSIKIAWESPQGQVSRYRVTYSSPEDGIRELFPAPDGEDDTAELQGLRPGSEYTVSVVALHDDMESQPLIGIQSTKRYKNRVASRKSRAKFKQLLQHYREVAAAKSSENDRLRLLLKESLKISQAVHAAHAEINEAGREVVGVGALKVPRNQDWLGVPRFAKFASFEAQGALANIAVDKANLDVEQLESIINFEKLTEWTGS

SEQ ID NO: 27 - protein, 169 aa, Artificial Sequence
  AnaxaZ13Mad5
MHHHHHHSTVHEILCKLSLEGDHSTPPSAYGSVKPYTNFDAEKRYKNRVASRKSRAKFKQLLQHYREVAAAKSSENDRLRLLLKESLKISQAVHAAHAEINEAGREVVGVGALKVPRNQDWLGVPRFAKFASFEAQGALANIAVDKANLDVEQLESIINFEKLTEWTGS

SEQ ID NO: 28 - protein, 169 aa, Artificial Sequence
  Z13Mad5Anaxa
MHHHHHHKRYKNRVASRKSRAKFKQLLQHYREVAAAKSSENDRLRLLLKESLKISQAVHAAHAEINEAGREVVGVGALKVPRNQDWLGVPRFAKFASFEAQGALANIAVDKANLDVEQLESIINFEKLTEWTGSSTVHEILCKLSLEGDHSTPPSAYGSVKPYTNFDAE

SEQ ID NO: 29 - protein, 157 aa, Artificial Sequence
  Z14Mad5Anaxa
MHHHHHHKRYKNRVASRKSRAKFKQLLQHYREVAAAKESLKISQAVHAAHAEINEAGREVVGVGALKVPRNQDWLGVPRFAKFASFEAQGALANIAVDKANLDVEQLESIINFEKLTEWTGSSTVHEILCKLSLEGDHSTPPSAYGSVKPYTNFDAE

SEQ ID NO: 30 - protein, 146 aa, Artificial Sequence
  Z18Mad5Anaxa
MHHHHHHREVAAAKSSENDRLRLLLKESLKISQAVHAAHAEINEAGREVVGVGALKVPRNQDWLGVPRFAKFASFEAQGALANIAVDKANLDVEQLESIINFEKLTEWTGSSTVHEILCKLSLEGDHSTPPSAYGSVKPYTNFDAE

SEQ ID NO: 31 - protein, 212 aa, Artificial Sequence
  EDAZ14Mad5
MHHHHHHNIDRPKGLAFTDVDVDSIKIAWESPQGQVSRYRVTYSSPEDGIRELFPAPDGEDDTAELQGLRPGSEYTVSVVALHDDMESQPLIGIQSTKRYKNRVASRKSRAKFKQLLQHYREVAAAKESLKISQAVHAAHAEINEAGREVVGVGALKVPRNQDWLGVPRFAKFASFEAQGALANIAVDKANLDVEQLESIINFEKLTEWTGS

SEQ ID NO: 32 - protein, 201 aa, Artificial Sequence
  EDAZ18Mad5
MHHHHHHNIDRPKGLAFTDVDVDSIKIAWESPQGQVSRYRVTYSSPEDGIRELFPAPDGEDDTAELQGLRPGSEYTVSVVALHDDMESQPLIGIQSTREVAAAKSSENDRLRLLLKESLKISQAVHAAHAEINEAGREVVGVGALKVPRNQDWLGVPRFAKFASFEAQGALANIAVDKANLDVEQLESIINFEKLTEWTGS

SEQ ID NO: 33 - protein, 116 aa, Artificial Sequence
  Z13Mad8Anaxa
KRYKNRVASRKSRAKFKQLLQHYREVAAAKSSENDRLRLLLKVTYHSPSYVYHQFERRAILNRLVQFIKDRISVVQALVLTSTVHEILCKLSLEGDHSTPPSAYGSVKPYTNFDAE

SEQ ID NO: 34 - protein, 182 aa, Artificial Sequence
  EDAMad5
MHHHHHHNIDRPKGLAFTDVDVDSIKIAWESPQGQVSRYRVTYSSPEDGIRELFPAPDGEDDTAELQGLRPGSEYTVSVVALHDDMESQPLIGIQSTESLKISQAVHAAHAEINEAGREVVGVGALKVPRNQDWLGVPRFAKFASFEAQGALANIAVDKANLDVEQLESIINFEKLTEWTGS

SEQ ID NO: 35 - protein, 8 aa, Artificial Sequence
  SIINFEKL OVACD8 peptide
SIINFEKL

SEQ ID NO: 36 - protein, 30 aa, Artificial Sequence
  Mad8
VTYHSPSYAYHQFERRAILNRLVQFIKDRI

SEQ ID NO: 37 - protein, 33 aa, Artificial Sequence
  Mad11
NYRIATFKNWPFLEDCAMEELTVSEFLKLDRQR

SEQ ID NO: 38 - protein, 17 aa, Artificial Sequence
  Mad9
HLELASMTNMELMSSIV

SEQ ID NO: 39 - protein, 50 aa, Artificial Sequence
  Mad12
LFRAAQLANDVVLQIMEHLELASMTNMELMSSIVVISASIIVFNLLELEG

SEQ ID NO: 40 - protein, 90 aa, Artificial Sequence
  EDA
NIDRPKGLAFTDVDVDSIKIAWESPQGQVSRYRVTYSSPEDGIRELFPAPDGEDDTAELQGLRPGSEYTVSVVALHDDMESQPLIGIQST

SEQ ID NO: 41 - protein, 116 aa, Artificial Sequence
  Z13Mad8Anaxa
KRYKNRVASRKSRAKFKQLLQHYREVAAAKSSENDRLRLLLKVTYHSPSYAYHQFERRAILNRLVQFIKDRISVVQALVLTSTVHEILCKLSLEGDHSTPPSAYGSVKPYTNFDAE

SEQ ID NO: 42 - protein, 110 aa, Artificial Sequence
  Z13Mad11Anaxa
KRYKNRVASRKSRAKFKQLLQHYREVAAAKSSENDRLRLLLKNYRIATFKNWPFLEDCAMEELTVSEFLKLDRQRSTVHEILCKLSLEGDHSTPPSAYGSVKPYTNFDAE

SEQ ID NO: 43 - protein, 94 aa, Artificial Sequence
  Z13Mad9Anaxa
KRYKNRVASRKSRAKFKQLLQHYREVAAAKSSENDRLRLLLKHLELASMTNMELMSSIVSTVHEILCKLSLEGDHSTPPSAYGSVKPYTNFDAE

SEQ ID NO: 44 - protein, 115 aa, Artificial Sequence
  TatFMad5Anaxa
RKKRRQRRRRVKRISQAVHAAHAEINEAGRRVKRKVPRNQDWLRVKRASFEAQGALANIAVDKARVKRSIINFEKLRVKRSTVHEILCKLSLEGDHSTPPSAYGSVKPYTNFDAE

SEQ ID NO: 45 - protein, 127 aa, Artificial Sequence
  Z13Mad12Anaxa
KRYKNRVASRKSRAKFKQLLQHYREVAAAKSSENDRLRLLLKLFRAAQLANDVVLQIMEHLELASMTNMELMSSIVVISASIIVFNLLELEGSTVHEILCKLSLEGDHSTPPSAYGSVKPYTNFDAE

SEQ ID NO: 46 - protein, 134 aa, Artificial Sequence
  Z13Mad5
MHHHHHHKRYKNRVASRKSRAKFKQLLQHYREVAAAKSSENDRLRLLLKESLKISQAVHAAHAEINEAGREVVGVGALKVPRNQDWLGVPRFAKFASFEAQGALANIAVDKANLDVEQLESIINFEKLTEWTGS

SEQ ID NO: 47 - protein, 35 aa, Artificial Sequence
  TLR peptide agonist: "Anaxa" sequence variant
STVHEILSKLSLEGDHSTPPSAYGSVKPYTNFDAE